European Patent Application EP 4 261 228 A1, published October 18, 2023. Title: ANTIBODY SPECIFICALLY BINDING TO STREP-TAG II TAG AND USE THEREOF. Applicant: BEIJING IMMUNOCHINA PHARMACEUTICALS CO.,LTD. BEIJING YIMIAOYILIAO CO.,LTD. The sequence listing filed with the application follows.

SEQUENCE LISTING (30 sequences)

SEQ ID NO: 1 - protein, 10 aa, Artificial Sequence
  VH-CDR1
GYTFTDYYMK

SEQ ID NO: 2 - protein, 17 aa, Artificial Sequence
  VH-CDR2
DINPNNGDTFYNQKFKG

SEQ ID NO: 3 - protein, 11 aa, Artificial Sequence
  VH-CDR3
YYGNSSPWFAY

SEQ ID NO: 4 - protein, 11 aa, Artificial Sequence
  VH-CDR3
YYGRSSPWFPY

SEQ ID NO: 5 - protein, 15 aa, Artificial Sequence
  VL-CDR1
KASQSVDYDGDSYMN

SEQ ID NO: 6 - protein, 15 aa, Artificial Sequence
  VL-CDR1
KASQSVDNSGDSYMN

SEQ ID NO: 7 - protein, 7 aa, Artificial Sequence
  VL-CDR2
AASNLQS

SEQ ID NO: 8 - protein, 7 aa, Artificial Sequence
  VL-CDR2
AASNLES

SEQ ID NO: 9 - protein, 9 aa, Artificial Sequence
  VL-CDR3
QQITEDPWT

SEQ ID NO: 10 - protein, 9 aa, Artificial Sequence
  VL-CDR3
QQINEDPWT

SEQ ID NO: 11 - protein, 25 aa, Artificial Sequence
  VH-FWR1
EVQLQQSGPELVKPGASVKMSCKAS

SEQ ID NO: 12 - protein, 14 aa, Artificial Sequence
  VH-FWR2
WVKQSHGKSLEWIG

SEQ ID NO: 13 - protein, 14 aa, Artificial Sequence
  VH-FWR2
WVKQSHGKRLEWIG

SEQ ID NO: 14 - protein, 32 aa, Artificial Sequence
  VH-FWR3
KATLTVDKSSSSAYMQLNSLTSEDSAVYYCAR

SEQ ID NO: 15 - protein, 32 aa, Artificial Sequence
  VH-FWR3
KATLTVDKSSSTAYMQLNSLTSEDSAVYYCAR

SEQ ID NO: 16 - protein, 11 aa, Artificial Sequence
  VH-FWR4
WGQGTLVTVSA

SEQ ID NO: 17 - protein, 23 aa, Artificial Sequence
  VL-FWR1
DIVLTQSPASLAVSLGQRATISC

SEQ ID NO: 18 - protein, 23 aa, Artificial Sequence
  VL-FWR1
DIVLTQSPASLGVSLGQRATISC

SEQ ID NO: 19 - protein, 15 aa, Artificial Sequence
  VL-FWR2
WYQQKPGQPPKLLIY

SEQ ID NO: 20 - protein, 32 aa, Artificial Sequence
  VL-FWR3
GIPARFSGSGSGTDFTLNIHPVEEEDTATYYC

SEQ ID NO: 21 - protein, 32 aa, Artificial Sequence
  VL-FWR3
GIPARFSGSGSGTDFTLNIHPVEEEDAATYYC

SEQ ID NO: 22 - protein, 10 aa, Artificial Sequence
  VL-FWR4
FGGRTKLEIK

SEQ ID NO: 23 - protein, 120 aa, Artificial Sequence
  Heavy Chain Variable Region
EVQLQQSGPELVKPGASVKMSCKASGYTFTDYYMKWVKQSHGKSLEWIGDINPNNGDTFYNQKFKGKATLTVDKSSSSAYMQLNSLTSEDSAVYYCARYYGNSSPWFAYWGQGTLVTVSA

SEQ ID NO: 24 - protein, 120 aa, Artificial Sequence
  Heavy Chain Variable Region
EVQLQQSGPELVKPGASVKMSCKASGYTFTDYYMKWVKQSHGKRLEWIGDINPNNGDTFYNQKFKGKATLTVDKSSSTAYMQLNSLTSEDSAVYYCARYYGRSSPWFPYWGQGTLVTVSA

SEQ ID NO: 25 - protein, 111 aa, Artificial Sequence
  Light Chain Variable Region
DIVLTQSPASLAVSLGQRATISCKASQSVDYDGDSYMNWYQQKPGQPPKLLIYAASNLQSGIPARFSGSGSGTDFTLNIHPVEEEDTATYYCQQITEDPWTFGGRTKLEIK

SEQ ID NO: 26 - protein, 111 aa, Artificial Sequence
  Light Chain Variable Region
DIVLTQSPASLGVSLGQRATISCKASQSVDNSGDSYMNWYQQKPGQPPKLLIYAASNLESGIPARFSGSGSGTDFTLNIHPVEEEDAATYYCQQINEDPWTFGGRTKLEIK

SEQ ID NO: 27 - protein, 444 aa, Artificial Sequence
  Heavy Chain
EVQLQQSGPELVKPGASVKMSCKASGYTFTDYYMKWVKQSHGKSLEWIGDINPNNGDTFYNQKFKGKATLTVDKSSSSAYMQLNSLTSEDSAVYYCARYYGNSSPWFAYWGQGTLVTVSAAKTTPPSVYPLAPGSAAQTNSMVTLGCLVKGYFPEPVTVTWNSGSLSSGVHTFPAVLQSDLYTLSSSVTVPSSPRPSETVTCNVAHPASSTKVDKKIVPRDCGCKPCICTVPEVSSVFIFPPKPKDVLTITLTPKVTCVVVDISKDDPEVQFSWFVDDVEVHTAQTQPREEQFNSTFRSVSELPIMHQDWLNGKEFKCRVNSAAFPAPIEKTISKTKGRPKAPQVYTIPPPKEQMAKDKVSLTCMITDFFPEDITVEWQWNGQPAENYKNTQPIMNTNGSYFVYSKLNVQKSNWEAGNTFTCSVLHEGLHNHHTEKSLSHSPGK

SEQ ID NO: 28 - protein, 218 aa, Artificial Sequence
  Light Chain
DIVLTQSPASLAVSLGQRATISCKASQSVDYDGDSYMNWYQQKPGQPPKLLIYAASNLQSGIPARFSGSGSGTDFTLNIHPVEEEDTATYYCQQITEDPWTFGGRTKLEIKRADAAPTVSIFPPSSEQLTSGGASVVCFLNNFYPKDINVKWKIDGSERQNGVLNSWTDQDSKDSTYSMSSTLTLTKDEYERHNSYTCEATHKTSTSPIVKSFNRNEC

SEQ ID NO: 29 - protein, 444 aa, Artificial Sequence
  Heavy Chain
EVQLQQSGPELVKPGASVKMSCKASGYTFTDYYMKWVKQSHGKRLEWIGDINPNNGDTFYNQKFKGKATLTVDKSSSTAYMQLNSLTSEDSAVYYCARYYGRSSPWFPYWGQGTLVTVSAAKTTPPSVYPLAPGSAAQTNSMVTLGCLVKGYFPEPVTVTWNSGSLSSGVHTFPAVLQSDLYTLSSSVTVPSSPRPSETVTCNVAHPASSTKVDKKIVPRDCGCKPCICTVPEVSSVFIFPPKPKDVLTITLTPKVTCVVVDISKDDPEVQFSWFVDDVEVHTAQTQPREEQFNSTFRSVSELPIMHQDWLNGKEFKCRVNSAAFPAPIEKTISKTKGRPKAPQVYTIPPPKEQMAKDKVSLTCMITDFFPEDITVEWQWNGQPAENYKNTQPIMNTNGSYFVYSKLNVQKSNWEAGNTFTCSVLHEGLHNHHTEKSLSHSPGK

SEQ ID NO: 30 - protein, 218 aa, Artificial Sequence
  Light Chain
DIVLTQSPASLGVSLGQRATISCKASQSVDNSGDSYMNWYQQKPGQPPKLLIYAASNLESGIPARFSGSGSGTDFTLNIHPVEEEDAATYYCQQINEDPWTFGGRTKLEIKRADAAPTVSIFPPSSEQLTSGGASVVCFLNNFYPKDINVKWKIDGSERQNGVLNSWTDQDSKDSTYSMSSTLTLTKDEYERHNSYTCEATHKTSTSPIVKSFNRNEC